European Patent Specification EP 3 765 055 B9, published September 27, 2023. Title: BACTERIAL-BINDING PEPTIDES FOR TREATMENT OF INFECTIOUS DISEASES AND RELATED INFLAMMATORY PROCESSES. Applicant: Institut d’investigacions Biomèdiques August Pi i Sunyer (IDIBAPS) Hospital Clinic de Barcelona. The sequence listing filed with the application follows.

SEQUENCE LISTING (39 sequences)

SEQ ID NO: 1 - protein, 11 aa, Artificial Sequence
  CD6.PD1
GTVEVRLEASW

SEQ ID NO: 2 - protein, 11 aa, Artificial Sequence
  CD6.PD2
GRVEMLEHGEW

SEQ ID NO: 3 - protein, 11 aa, Artificial Sequence
  CD6.PD3
GQVEVHFRGVW

SEQ ID NO: 4 - protein, 373 aa, Homo sapiens
  hCD6
DQLNTSSAESELWEPGERLPVRLTNGSSSCSGTVEVRLEASWEPACGALWDSRAAEAVCRALGCGGAEAASQLAPPTPELPPPPAAGNTSVAANATLAGAPALLCSGAEWRLCEVVEHACRSDGRRARVTCAENRALRLVDGGGACAGRVEMLEHGEWGSVCDDTWDLEDAHVVCRQLGCGWAVQALPGLHFTPGRGPIHRDQVNCSGAEAYLWDCPGLPGQHYCGHKEDAGVVCSEHQSWRLTGGADRCEGQVEVHFRGVWNTVCDSEWYPSEAKVLCQSLGCGTAVERPKGLPHSLSGRMYYSCNGEELTLSNCSWRFNNSNLCSQSLAARVLCSASRSLHNLSTPEVPASVQTVTIESSVTVKIENKESR

SEQ ID NO: 5 - DNA, 1122 bp, Homo sapiens
  hCD6
gaccagctcaacaccagcagtgcagagagtgagctctgggagccaggggagcggcttccggtccgtctgacaaacgggagcagcagctgcagcgggacggtggaggtgcggctcgaggcgtcctgggagcccgcgtgcggggcgctctgggacagccgcgccgccgaggccgtgtgccgagcactgggctgcggcggggcggaggccgcctctcagctcgccccgccgacccctgagctgccgcccccgcctgcagccgggaacaccagcgtagcagctaatgccactctggccggggcgcccgccctcctgtgcagcggcgccgagtggcggctctgcgaggtggtggagcacgcgtgccgcagcgacgggaggcgggcccgtgtcacctgtgcagagaaccgcgcgctgcgcctggtggacggtggcggcgcctgcgccggccgcgtggagatgctggagcatggcgagtggggatcagtgtgcgatgacacttgggacctggaggacgcccacgtggtgtgcaggcaactgggctgcggctgggcagtccaggccctgcccggcttgcacttcacgcccggccgcgggcctatccaccgggaccaggtgaactgctcgggggccgaagcttacctgtgggactgcccggggctgccaggacagcactactgcggccacaaagaggacgcgggcgtggtgtgctcagagcaccagtcctggcgcctgacagggggcgctgaccgctgcgaggggcaggtggaggtacacttccgaggggtctggaacacagtgtgtgacagtgagtggtacccatcggaggccaaggtgctctgccagtccttgggctgtggaactgcggttgagaggcccaaggggctgccccactccttgtccggcaggatgtactactcatgcaatggggaggagctcaccctctccaactgctcctggcggttcaacaactccaacctctgcagccagtcgctggcagccagggtcctctgctcagcttcccggagtttgcacaatctgtccactcccgaagtccctgcaagtgttcagacagtcactatagaatcttctgtgacagtgaaaatagagaacaaggaatctcggtag

SEQ ID NO: 6 - protein, 11 aa, Artificial Sequence
  CD5.PD1
GQLEVYLKDGW

SEQ ID NO: 7 - protein, 11 aa, Artificial Sequence
  CD5.PD2
GVVEFYSGSLG

SEQ ID NO: 8 - protein, 11 aa, Artificial Sequence
  DMBT-1.pbs1
GRVEVLYRGSW

SEQ ID NO: 9 - protein, 11 aa, Artificial Sequence
  CD6 Pcon
GRVEVLFRGSW

SEQ ID NO: 10 - protein, 373 aa, Artificial Sequence
  rshCD6
DQLNTSSAESELWEPGERLPVRLTNGSSSCSGTVEVRLEASWEPACGALWDSRAAEAVCRALGCGGAEAASQLAPPTPELPPPPAAGNTSVAANATLAGAPALLCSGAEWRLCEVVEHACRSDGRRARVTCAENRALRLVDGGGACAGRVEMLEHGEWGSVCDDTWDLEDAHVVCRQLGCGWAVQALPGLHFTPGRGPIHRDQVNCSGAEAYLWDCPGLPGQHYCGHKEDAGAVCSEHQSWRLTGGADRCEGQVEVHFRGVWNTVCDSEWYPSEAKVLCQSLGCGTAVERPKGLPHSLSGRMYYSCNGEELTLSNCSWRFNNSNLCSQSLAARVLCSASRSLHNLSTPEVPASVQTVTIESSVTVKIENKESR

SEQ ID NO: 11 - protein, 334 aa, Artificial Sequence
  rshCD5
RLTRSNSKCQGQLEVYLKDGWHMVCSQSWGRSSKQWEDPSQASKVCQRLNCGVPLSLGPFLVTYTPQSSIICYGQLGSFSNCSHSRNDMCHSLGLTCLEPQKTTPPTTRPPPTTTPEPTAPPRLQLVAQSGGQHCAGVVEFYSGSLGGTISYEAQDKTQDLENFLCNNLQCGSFLKHLPETEAGRAQDPGEPREHQPLPIQWKIQNSSCTSLEHCFRKIKPQKSGRVLALLCSGFQPKVQSRLVGGSSICEGTVEVRQGAQWAALCDSSSARSSLRWEEVCREQQCGSVNSYRVLDAGDPTSRGLFCPHQKLSQCHELWERNSYCKKVFVTCQD

SEQ ID NO: 12 - protein, 609 aa, Homo sapiens [sequence omitted]

SEQ ID NO: 13 - protein, 17 aa, Artificial Sequence
  Peptide
CSGTVEVRLEASWEPAC

SEQ ID NO: 14 - protein, 15 aa, Artificial Sequence
  Peptide
SGTVEVRLEASWEPA

SEQ ID NO: 15 - protein, 14 aa, Artificial Sequence
  Peptide
SGTVEVRLEASWEP

SEQ ID NO: 16 - protein, 13 aa, Artificial Sequence
  Peptide
SGTVEVRLEASWE

SEQ ID NO: 17 - protein, 12 aa, Artificial Sequence
  Peptide
SGTVEVRLEASW

SEQ ID NO: 18 - protein, 14 aa, Artificial Sequence
  Peptide
GTVEVRLEASWEPA

SEQ ID NO: 19 - protein, 13 aa, Artificial Sequence
  Peptide
GTVEVRLEASWEP

SEQ ID NO: 20 - protein, 12 aa, Artificial Sequence
  Peptide
GTVEVRLEASWE

SEQ ID NO: 21 - protein, 17 aa, Artificial Sequence
  Peptide
CAGRVEMLEHGEWGSVC

SEQ ID NO: 22 - protein, 15 aa, Artificial Sequence
  Peptide
AGRVEMLEHGEWGSV

SEQ ID NO: 23 - protein, 14 aa, Artificial Sequence
  Peptide
AGRVEMLEHGEWGS

SEQ ID NO: 24 - protein, 13 aa, Artificial Sequence
  Peptide
AGRVEMLEHGEWG

SEQ ID NO: 25 - protein, 12 aa, Artificial Sequence
  Peptide
AGRVEMLEHGEW

SEQ ID NO: 26 - protein, 14 aa, Artificial Sequence
  Peptide
GRVEMLEHGEWGSV

SEQ ID NO: 27 - protein, 13 aa, Artificial Sequence
  Peptide
GRVEMLEHGEWGS

SEQ ID NO: 28 - protein, 12 aa, Artificial Sequence
  Peptide
GRVEMLEHGEWG

SEQ ID NO: 29 - protein, 17 aa, Artificial Sequence
  Peptide
CEGQVEVHFRGVWNTVC

SEQ ID NO: 30 - protein, 15 aa, Artificial Sequence
  Peptide
EGQVEVHFRGVWNTV

SEQ ID NO: 31 - protein, 14 aa, Artificial Sequence
  Peptide
EGQVEVHFRGVWNT

SEQ ID NO: 32 - protein, 13 aa, Artificial Sequence
  Peptide
EGQVEVHFRGVWN

SEQ ID NO: 33 - protein, 12 aa, Artificial Sequence
  Peptide
EGQVEVHFRGVW

SEQ ID NO: 34 - protein, 14 aa, Artificial Sequence
  Peptide
GQVEVHFRGVWNTV

SEQ ID NO: 35 - protein, 13 aa, Artificial Sequence
  Peptide
GQVEVHFRGVWNT

SEQ ID NO: 36 - protein, 12 aa, Artificial Sequence
  Peptide
GQVEVHFRGVWN

SEQ ID NO: 37 - protein, 17 aa, Artificial Sequence
  DISULFID join(1,17): join(1,17)
  13c
CSGTVEVRLEASWEPAC

SEQ ID NO: 38 - protein, 17 aa, Artificial Sequence
  DISULFID join(1,17): join(1,17)
  21c
CAGRVEMLEHGEWGSVC

SEQ ID NO: 39 - protein, 17 aa, Artificial Sequence
  DISULFID join(1,17): join(1,17)
  29c
CEGQVEVHFRGVWNTVC